European Patent Specification EP 3 414 328 B1, published January 10, 2024. Title: Novel enymes for trimming of glycoproteins. Applicant: Synaffix B.V. The sequence listing filed with the application follows.

SEQUENCE LISTING (33 sequences)

SEQ ID NO: 1 - protein, 1258 aa, Artificial sequence
  EndoS-EndoH
MPSIDSLHYLSENSKKEFKEELSKAGQESQKVKEILAKAQQADKQAQELAKMKIPEKIPMKPLHGPLYGGYFRTWHDKTSDPTEKDKVNSMGELPKEVDLAFIFHDWTKDYSLFWKELATKHVPKLNKQGTRVIRTIPWRFLAGGDNSGIAEDTSKYPNTPEGNKALAKAIVDEYVYKYNLDGLDVDVEHDSIPKVDKKEDTAGVERSIQVFEEIGKLIGPKGVDKSRLFIMDSTYMADKNPLIERGAPYINLLLVQVYGSQGEKGGWEPVSNRPEKTMEERWQGYSKYIRPEQYMIGFSFYEENAQEGNLWYDINSRKDEDKANGINTDITGTRAERYARWQPKTGGVKGGIFSYAIDRDGVAHQPKKYAKQKEFKDATDNIFHSDYSVSKALKTVMLKDKSYDLIDEKDFPDKALREAVMAQVGTRKGDLERFNGTLRLDNPAIQSLEGLNKFKKLAQLDLIGLSRITKLDRSVLPANMKPGKDTLETVLETYKKDNKEEPATIPPVSLKVSGLTGLKELDLSGFDRETLAGLDAATLTSLEKVDISGNKLDLAPGTENRQIFDTMLSTISNHVGSNEQTVKFDKQKPTGHYPDTYGKTSLRLPVANEKVDLQSQLLFGTVTNQGTLINSEADYKAYQNHKIAGRSFVDSNYHYNNFKVSYENYTVKVTDSTLGTTTDKTLATDKEETYKVDFFSPADKTKAVHTAKVIVGDEKTMMVNLAEGATVIGGSADPVNARKVFDGQLGSETDNISLGWDSKQSIIFKLKEDGLIKHWRFFNDSARNPETTNKPIQEASLQIFNIKDYNLDNLLENPNKFDDEKYWITVDTYSAQGERATAFSNTLNNITSKYWRVVFDTKGDRYSSPVVPELQILGYPLPNADTIMKTVTTAKELSQQKDKFSQKMLDELKIKEMALETSLNSKIFDVTAINANAGVLKDCIEKRQLLKKGGGGSGGGGSGGGGSHHHHHHEFGGGGSGGGGSGGGGSAPAPVKQGPTSVAYVEVNNNSMLNVGKYTLADGGGNAFDVAVIFAANINYDTGTKTAYLHFNENVQRVLDNAVTQIRPLQQQGIKVLLSVLGNHQGAGFANFPSQQAASAFAKQLSDAVAKYGLDGVDFDDEYAEYGNNGTAQPNDSSFVHLVTALRANMPDKIISLYNIGPAASRLSYGGVDVSDKFDYAWNPYYGTWQVPGIALPKAQLSPAAVEIGRTSRSTVADLARRTVDEGYGVYLTYNLDGGDRTADVSAFTRELYGSEAVRTP

SEQ ID NO: 2 - protein, 1256 aa, Artificial sequence
  EndoS-EndoH
MPSIDSLHYLSENSKKEFKEELSKAGQESQKVKEILAKAQQADKQAQELAKMKIPEKIPMKPLHGPLYGGYFRTWHDKTSDPTEKDKVNSMGELPKEVDLAFIFHDWTKDYSLFWKELATKHVPKLNKQGTRVIRTIPWRFLAGGDNSGIAEDTSKYPNTPEGNKALAKAIVDEYVYKYNLDGLDVDVEHDSIPKVDKKEDTAGVERSIQVFEEIGKLIGPKGVDKSRLFIMDSTYMADKNPLIERGAPYINLLLVQVYGSQGEKGGWEPVSNRPEKTMEERWQGYSKYIRPEQYMIGFSFYEENAQEGNLWYDINSRKDEDKANGINTDITGTRAERYARWQPKTGGVKGGIFSYAIDRDGVAHQPKKYAKQKEFKDATDNIFHSDYSVSKALKTVMLKDKSYDLIDEKDFPDKALREAVMAQVGTRKGDLERFNGTLRLDNPAIQSLEGLNKFKKLAQLDLIGLSRITKLDRSVLPANMKPGKDTLETVLETYKKDNKEEPATIPPVSLKVSGLTGLKELDLSGFDRETLAGLDAATLTSLEKVDISGNKLDLAPGTENRQIFDTMLSTISNHVGSNEQTVKFDKQKPTGHYPDTYGKTSLRLPVANEKVDLQSQLLFGTVTNQGTLINSEADYKAYQNHKIAGRSFVDSNYHYNNFKVSYENYTVKVTDSTLGTTTDKTLATDKEETYKVDFFSPADKTKAVHTAKVIVGDEKTMMVNLAEGATVIGGSADPVNARKVFDGQLGSETDNISLGWDSKQSIIFKLKEDGLIKHWRFFNDSARNPETTNKPIQEASLQIFNIKDYNLDNLLENPNKFDDEKYWITVDTYSAQGERATAFSNTLNNITSKYWRVVFDTKGDRYSSPVVPELQILGYPLPNADTIMKTVTTAKELSQQKDKFSQKMLDELKIKEMALETSLNSKIFDVTAINANAGVLKDCIEKRQLLKKGGGGSGGGGSGGGGSHHHHHHGGGGSGGGGSGGGGSAPAPVKQGPTSVAYVEVNNNSMLNVGKYTLADGGGNAFDVAVIFAANINYDTGTKTAYLHFNENVQRVLDNAVTQIRPLQQQGIKVLLSVLGNHQGAGFANFPSQQAASAFAKQLSDAVAKYGLDGVDFDDEYAEYGNNGTAQPNDSSFVHLVTALRANMPDKIISLYNIGPAASRLSYGGVDVSDKFDYAWNPYYGTWQVPGIALPKAQLSPAAVEIGRTSRSTVADLARRTVDEGYGVYLTYNLDGGDRTADVSAFTRELYGSEAVRTP

SEQ ID NO: 3 - protein, 410 aa, Artificial sequence
  His-TnGalNAcT(33-421)
MGSSHHHHHHSSGLVPRGSHMSPLRTYLYTPLYNATQPTLRNVERLAANWPKKIPSNYIEDSEEYSIKNISLSNHTTRASVVHPPSSITETASKLDKNMTIQDGAFAMISPTPLLITKLMDSIKSYVTTEDGVKKAEAVVTLPLCDSMPPDLGPITLNKTELELEWVEKKFPEVEWGGRYSPPNCTARHRVAIIVPYRDRQQHLAIFLNHMHPFLMKQQIEYGIFIVEQEGNKDFNRAKLMNVGFVESQKLVAEGWQCFVFHDIDLLPLDTRNLYSCPRQPRHMSASIDKLHFKLPYEDIFGGVSAMTLEQFTRVNGFSNKYWGWGGEDDDMSYRLKKINYHIARYKMSIARYAMLDHKKSTPNPKRYQLLSQTSKTFQKDGLSTLEYELVQVVQYHLYTHILVNIDERS

SEQ ID NO: 4 - protein, 949 aa, Artificial sequence
  EndoS
MPSIDSLHYLSENSKKEFKEELSKAGQESQKVKEILAKAQQADKQAQELAKMKIPEKIPMKPLHGPLYGGYFRTWHDKTSDPTEKDKVNSMGELPKEVDLAFIFHDWTKDYSLFWKELATKHVPKLNKQGTRVIRTIPWRFLAGGDNSGIAEDTSKYPNTPEGNKALAKAIVDEYVYKYNLDGLDVDVEHDSIPKVDKKEDTAGVERSIQVFEEIGKLIGPKGVDKSRLFIMDSTYMADKNPLIERGAPYINLLLVQVYGSQGEKGGWEPVSNRPEKTMEERWQGYSKYIRPEQYMIGFSFYEENAQEGNLWYDINSRKDEDKANGINTDITGTRAERYARWQPKTGGVKGGIFSYAIDRDGVAHQPKKYAKQKEFKDATDNIFHSDYSVSKALKTVMLKDKSYDLIDEKDFPDKALREAVMAQVGTRKGDLERFNGTLRLDNPAIQSLEGLNKFKKLAQLDLIGLSRITKLDRSVLPANMKPGKDTLETVLETYKKDNKEEPATIPPVSLKVSGLTGLKELDLSGFDRETLAGLDAATLTSLEKVDISGNKLDLAPGTENRQIFDTMLSTISNHVGSNEQTVKFDKQKPTGHYPDTYGKTSLRLPVANEKVDLQSQLLFGTVTNQGTLINSEADYKAYQNHKIAGRSFVDSNYHYNNFKVSYENYTVKVTDSTLGTTTDKTLATDKEETYKVDFFSPADKTKAVHTAKVIVGDEKTMMVNLAEGATVIGGSADPVNARKVFDGQLGSETDNISLGWDSKQSIIFKLKEDGLIKHWRFFNDSARNPETTNKPIQEASLQIFNIKDYNLDNLLENPNKFDDEKYWITVDTYSAQGERATAFSNTLNNITSKYWRVVFDTKGDRYSSPVVPELQILGYPLPNADTIMKTVTTAKELSQQKDKFSQKMLDELKIKEMALETSLNSKIFDVTAINANAGVLKDCIEKRQLLKK

SEQ ID NO: 5 - protein, 969 aa, Artificial sequence
  EndoS 2
MGSSHHHHHHSSGLVPRGSHMPSIDSLHYLSENSKKEFKEELSKAGQESQKVKEILAKAQQADKQAQELAKMKIPEKIPMKPLHGPLYGGYFRTWHDKTSDPTEKDKVNSMGELPKEVDLAFIFHDWTKDYSLFWKELATKHVPKLNKQGTRVIRTIPWRFLAGGDNSGIAEDTSKYPNTPEGNKALAKAIVDEYVYKYNLDGLDVDVEHDSIPKVDKKEDTAGVERSIQVFEEIGKLIGPKGVDKSRLFIMDSTYMADKNPLIERGAPYINLLLVQVYGSQGEKGGWEPVSNRPEKTMEERWQGYSKYIRPEQYMIGFSFYEENAQEGNLWYDINSRKDEDKANGINTDITGTRAERYARWQPKTGGVKGGIFSYAIDRDGVAHQPKKYAKQKEFKDATDNIFHSDYSVSKALKTVMLKDKSYDLIDEKDFPDKALREAVMAQVGTRKGDLERFNGTLRLDNPAIQSLEGLNKFKKLAQLDLIGLSRITKLDRSVLPANMKPGKDTLETVLETYKKDNKEEPATIPPVSLKVSGLTGLKELDLSGFDRETLAGLDAATLTSLEKVDISGNKLDLAPGTENRQIFDTMLSTISNHVGSNEQTVKFDKQKPTGHYPDTYGKTSLRLPVANEKVDLQSQLLFGTVTNQGTLINSEADYKAYQNHKIAGRSFVDSNYHYNNFKVSYENYTVKVTDSTLGTTTDKTLATDKEETYKVDFFSPADKTKAVHTAKVIVGDEKTMMVNLAEGATVIGGSADPVNARKVFDGQLGSETDNISLGWDSKQSIIFKLKEDGLIKHWRFFNDSARNPETTNKPIQEASLQIFNIKDYNLDNLLENPNKFDDEKYWITVDTYSAQGERATAFSNTLNNITSKYWRVVFDTKGDRYSSPVVPELQILGYPLPNADTIMKTVTTAKELSQQKDKFSQKMLDELKIKEMALETSLNSKIFDVTAINANAGVLKDCIEKRQLLKK

SEQ ID NO: 6 - protein, 271 aa, Artificial sequence
  EndoH
APAPVKQGPTSVAYVEVNNNSMLNVGKYTLADGGGNAFDVAVIFAANINYDTGTKTAYLHFNENVQRVLDNAVTQIRPLQQQGIKVLLSVLGNHQGAGFANFPSQQAASAFAKQLSDAVAKYGLDGVDFDDEYAEYGNNGTAQPNDSSFVHLVTALRANMPDKIISLYNIGPAASRLSYGGVDVSDKFDYAWNPYYGTWQVPGIALPKAQLSPAAVEIGRTSRSTVADLARRTVDEGYGVYLTYNLDGGDRTADVSAFTRELYGSEAVRTP

SEQ ID NO: 7 - protein, 289 aa, Artificial sequence
  EndoF1
AVTGTTKANIKLFSFTEVNDTNPLNNLNFTLKNSGKPLVDMVVLFSANINYDAANDKVFVSNNPNVQHLLTNRAKYLKPLQDKGIKVILSILGNHDRSGIANLSTARAKAFAQELKNTCDLYNLDGVFFDDEYSAYQTPPPSGFVTPSNNAAARLAYETKQAMPNKLVTVYVYSRTSSFPTAVDGVNAGSYVDYAIHDYGGSYDLATNYPGLAKSGMVMSSQEFNQGRYATAQALRNIVTKGYGGHMIFAMDPNRSNFTSGQLPALKLIAKELYGDELVYSNTPYSKDW

SEQ ID NO: 8 - protein, 291 aa, Artificial sequence
  EndoF2
MAVNLSNLIAYKNSDHQISAGYYRTWRDSATASGNLPSMRWLPDSLDMVMVFPDYTPPENAYWNTLKTNYVPYLHKRGTKVIITLGDLNSATTTGGQDSIGYSSWAKGIYDKWVGEYNLDGIDIDIESSPSGATLTKFVAATKALSKYFGPKSGTGKTFVYDTNQNPTNFFIQTAPRYNYVFLQAYGRSTTNLTTVSGLYAPYISMKQFLPGFSFYEENGYPGNYWNDVRYPQNGTGRAYDYARWQPATGKKGGVFSYAIERDAPLTSSNDNTLRAPNFRVTKDLIKIMNP

SEQ ID NO: 9 - protein, 291 aa, Artificial sequence
  EndoF3
MATALAGSNGVCIAYYITDGRNPTFKLKDIPDKVDMVILFGLKYWSLQDTTKLPGGTGMMGSFKSYKDLDTQIRSLQSRGIKVLQNIDDDVSWQSSKPGGFASAAAYGDAIKSIVIDKWKLDGISLDIEHSGAKPNPIPTFPGYAATGYNGWYSGSMAATPAFLNVISELTKYFGTTAPNNKQLQIASGIDVYAWNKIMENFRNNFNYIQLQSYGANVSRTQLMMNYATGTNKIPASKMVFGAYAEGGTNQANDVEVAKWTPTQGAKGGMMIYTYNSNVSYANAVRDAVKN

SEQ ID NO: 10 - protein, 273 aa, Artificial sequence
  EfEndo18A
ASTVTPKTVMYVEVNNHDFNNVGKYTLAGTNQPAFDMGIIFAANINYDTVNKKPYLYLNERVQQTLNEAETQIRPVQARGTKVLLSILGNHEGAGFANFPTYESADAFAAQLEQVVNTYHLDGIDFDDEYAEYGKNGTPQPNNSSFIWLLQALRNRLGNDKLITFYNIGPAAANSSANPQMSSLIDYAWNPYYSTWNPPQIAGMPASRLGASAVEVGVNQNLAAQYAKRTKAEQYGIYLMYNLPGKDSSAYISAATQELYGRKTNYSPTVPTP

SEQ ID NO: 11 - protein, 38 aa, Artificial sequence
  linker
GGGGSGGGGSGGGGSHHHHHHEFGGGGSGGGGSGGGGS

SEQ ID NO: 12 - protein, 36 aa, Artificial sequence
  linker
GGGGSGGGGSGGGGSHHHHHHGGGGSGGGGSGGGGS

SEQ ID NO: 13 - protein, 602 aa, Artificial sequence
  EndoF3-EfEndo18A
MATALAGSNGVCIAYYITDGRNPTFKLKDIPDKVDMVILFGLKYWSLQDTTKLPGGTGMMGSFKSYKDLDTQIRSLQSRGIKVLQNIDDDVSWQSSKPGGFASAAAYGDAIKSIVIDKWKLDGISLDIEHSGAKPNPIPTFPGYAATGYNGWYSGSMAATPAFLNVISELTKYFGTTAPNNKQLQIASGIDVYAWNKIMENFRNNFNYIQLQSYGANVSRTQLMMNYATGTNKIPASKMVFGAYAEGGTNQANDVEVAKWTPTQGAKGGMMIYTYNSNVSYANAVRDAVKNGGGGSGGGGSGGGGSHHHHHHEFGGGGSGGGGSGGGGSASTVTPKTVMYVEVNNHDFNNVGKYTLAGTNQPAFDMGIIFAANINYDTVNKKPYLYLNERVQQTLNEAETQIRPVQARGTKVLLSILGNHEGAGFANFPTYESADAFAAQLEQVVNTYHLDGIDFDDEYAEYGKNGTPQPNNSSFIWLLQALRNRLGNDKLITFYNIGPAAANSSANPQMSSLIDYAWNPYYSTWNPPQIAGMPASRLGASAVEVGVNQNLAAQYAKRTKAEQYGIYLMYNLPGKDSSAYISAATQELYGRKTNYSPTVPTP

SEQ ID NO: 14 - protein, 602 aa, Artificial sequence
  EndoF2-EfEndo18A
MAVNLSNLIAYKNSDHQISAGYYRTWRDSATASGNLPSMRWLPDSLDMVMVFPDYTPPENAYWNTLKTNYVPYLHKRGTKVIITLGDLNSATTTGGQDSIGYSSWAKGIYDKWVGEYNLDGIDIDIESSPSGATLTKFVAATKALSKYFGPKSGTGKTFVYDTNQNPTNFFIQTAPRYNYVFLQAYGRSTTNLTTVSGLYAPYISMKQFLPGFSFYEENGYPGNYWNDVRYPQNGTGRAYDYARWQPATGKKGGVFSYAIERDAPLTSSNDNTLRAPNFRVTKDLIKIMNPGGGGSGGGGSGGGGSHHHHHHEFGGGGSGGGGSGGGGSASTVTPKTVMYVEVNNHDFNNVGKYTLAGTNQPAFDMGIIFAANINYDTVNKKPYLYLNERVQQTLNEAETQIRPVQARGTKVLLSILGNHEGAGFANFPTYESADAFAAQLEQVVNTYHLDGIDFDDEYAEYGKNGTPQPNNSSFIWLLQALRNRLGNDKLITFYNIGPAAANSSANPQMSSLIDYAWNPYYSTWNPPQIAGMPASRLGASAVEVGVNQNLAAQYAKRTKAEQYGIYLMYNLPGKDSSAYISAATQELYGRKTNYSPTVPTP

SEQ ID NO: 15 - protein, 1260 aa, Artificial sequence
  EndoS-EfEndo18A
MPSIDSLHYLSENSKKEFKEELSKAGQESQKVKEILAKAQQADKQAQELAKMKIPEKIPMKPLHGPLYGGYFRTWHDKTSDPTEKDKVNSMGELPKEVDLAFIFHDWTKDYSLFWKELATKHVPKLNKQGTRVIRTIPWRFLAGGDNSGIAEDTSKYPNTPEGNKALAKAIVDEYVYKYNLDGLDVDVEHDSIPKVDKKEDTAGVERSIQVFEEIGKLIGPKGVDKSRLFIMDSTYMADKNPLIERGAPYINLLLVQVYGSQGEKGGWEPVSNRPEKTMEERWQGYSKYIRPEQYMIGFSFYEENAQEGNLWYDINSRKDEDKANGINTDITGTRAERYARWQPKTGGVKGGIFSYAIDRDGVAHQPKKYAKQKEFKDATDNIFHSDYSVSKALKTVMLKDKSYDLIDEKDFPDKALREAVMAQVGTRKGDLERFNGTLRLDNPAIQSLEGLNKFKKLAQLDLIGLSRITKLDRSVLPANMKPGKDTLETVLETYKKDNKEEPATIPPVSLKVSGLTGLKELDLSGFDRETLAGLDAATLTSLEKVDISGNKLDLAPGTENRQIFDTMLSTISNHVGSNEQTVKFDKQKPTGHYPDTYGKTSLRLPVANEKVDLQSQLLFGTVTNQGTLINSEADYKAYQNHKIAGRSFVDSNYHYNNFKVSYENYTVKVTDSTLGTTTDKTLATDKEETYKVDFFSPADKTKAVHTAKVIVGDEKTMMVNLAEGATVIGGSADPVNARKVFDGQLGSETDNISLGWDSKQSIIFKLKEDGLIKHWRFFNDSARNPETTNKPIQEASLQIFNIKDYNLDNLLENPNKFDDEKYWITVDTYSAQGERATAFSNTLNNITSKYWRVVFDTKGDRYSSPVVPELQILGYPLPNADTIMKTVTTAKELSQQKDKFSQKMLDELKIKEMALETSLNSKIFDVTAINANAGVLKDCIEKRQLLKKGGGGSGGGGSGGGGSHHHHHHEFGGGGSGGGGSGGGGSASTVTPKTVMYVEVNNHDFNNVGKYTLAGTNQPAFDMGIIFAANINYDTVNKKPYLYLNERVQQTLNEAETQIRPVQARGTKVLLSILGNHEGAGFANFPTYESADAFAAQLEQVVNTYHLDGIDFDDEYAEYGKNGTPQPNNSSFIWLLQALRNRLGNDKLITFYNIGPAAANSSANPQMSSLIDYAWNPYYSTWNPPQIAGMPASRLGASAVEVGVNQNLAAQYAKRTKAEQYGIYLMYNLPGKDSSAYISAATQELYGRKTNYSPTVPTP

SEQ ID NO: 16 - protein, 618 aa, Artificial sequence
  EndoF3-EndoF1
MATALAGSNGVCIAYYITDGRNPTFKLKDIPDKVDMVILFGLKYWSLQDTTKLPGGTGMMGSFKSYKDLDTQIRSLQSRGIKVLQNIDDDVSWQSSKPGGFASAAAYGDAIKSIVIDKWKLDGISLDIEHSGAKPNPIPTFPGYAATGYNGWYSGSMAATPAFLNVISELTKYFGTTAPNNKQLQIASGIDVYAWNKIMENFRNNFNYIQLQSYGANVSRTQLMMNYATGTNKIPASKMVFGAYAEGGTNQANDVEVAKWTPTQGAKGGMMIYTYNSNVSYANAVRDAVKNGGGGSGGGGSGGGGSHHHHHHEFGGGGSGGGGSGGGGSAVTGTTKANIKLFSFTEVNDTNPLNNLNFTLKNSGKPLVDMVVLFSANINYDAANDKVFVSNNPNVQHLLTNRAKYLKPLQDKGIKVILSILGNHDRSGIANLSTARAKAFAQELKNTCDLYNLDGVFFDDEYSAYQTPPPSGFVTPSNNAAARLAYETKQAMPNKLVTVYVYSRTSSFPTAVDGVNAGSYVDYAIHDYGGSYDLATNYPGLAKSGMVMSSQEFNQGRYATAQALRNIVTKGYGGHMIFAMDPNRSNFTSGQLPALKLIAKELYGDELVYSNTPYSKDW

SEQ ID NO: 17 - protein, 618 aa, Artificial sequence
  EndoF2-EndoF1
MAVNLSNLIAYKNSDHQISAGYYRTWRDSATASGNLPSMRWLPDSLDMVMVFPDYTPPENAYWNTLKTNYVPYLHKRGTKVIITLGDLNSATTTGGQDSIGYSSWAKGIYDKWVGEYNLDGIDIDIESSPSGATLTKFVAATKALSKYFGPKSGTGKTFVYDTNQNPTNFFIQTAPRYNYVFLQAYGRSTTNLTTVSGLYAPYISMKQFLPGFSFYEENGYPGNYWNDVRYPQNGTGRAYDYARWQPATGKKGGVFSYAIERDAPLTSSNDNTLRAPNFRVTKDLIKIMNPGGGGSGGGGSGGGGSHHHHHHEFGGGGSGGGGSGGGGSAVTGTTKANIKLFSFTEVNDTNPLNNLNFTLKNSGKPLVDMVVLFSANINYDAANDKVFVSNNPNVQHLLTNRAKYLKPLQDKGIKVILSILGNHDRSGIANLSTARAKAFAQELKNTCDLYNLDGVFFDDEYSAYQTPPPSGFVTPSNNAAARLAYETKQAMPNKLVTVYVYSRTSSFPTAVDGVNAGSYVDYAIHDYGGSYDLATNYPGLAKSGMVMSSQEFNQGRYATAQALRNIVTKGYGGHMIFAMDPNRSNFTSGQLPALKLIAKELYGDELVYSNTPYSKDW

SEQ ID NO: 18 - protein, 1276 aa, Artificial sequence
  EndoS-EndoF1
MPSIDSLHYLSENSKKEFKEELSKAGQESQKVKEILAKAQQADKQAQELAKMKIPEKIPMKPLHGPLYGGYFRTWHDKTSDPTEKDKVNSMGELPKEVDLAFIFHDWTKDYSLFWKELATKHVPKLNKQGTRVIRTIPWRFLAGGDNSGIAEDTSKYPNTPEGNKALAKAIVDEYVYKYNLDGLDVDVEHDSIPKVDKKEDTAGVERSIQVFEEIGKLIGPKGVDKSRLFIMDSTYMADKNPLIERGAPYINLLLVQVYGSQGEKGGWEPVSNRPEKTMEERWQGYSKYIRPEQYMIGFSFYEENAQEGNLWYDINSRKDEDKANGINTDITGTRAERYARWQPKTGGVKGGIFSYAIDRDGVAHQPKKYAKQKEFKDATDNIFHSDYSVSKALKTVMLKDKSYDLIDEKDFPDKALREAVMAQVGTRKGDLERFNGTLRLDNPAIQSLEGLNKFKKLAQLDLIGLSRITKLDRSVLPANMKPGKDTLETVLETYKKDNKEEPATIPPVSLKVSGLTGLKELDLSGFDRETLAGLDAATLTSLEKVDISGNKLDLAPGTENRQIFDTMLSTISNHVGSNEQTVKFDKQKPTGHYPDTYGKTSLRLPVANEKVDLQSQLLFGTVTNQGTLINSEADYKAYQNHKIAGRSFVDSNYHYNNFKVSYENYTVKVTDSTLGTTTDKTLATDKEETYKVDFFSPADKTKAVHTAKVIVGDEKTMMVNLAEGATVIGGSADPVNARKVFDGQLGSETDNISLGWDSKQSIIFKLKEDGLIKHWRFFNDSARNPETTNKPIQEASLQIFNIKDYNLDNLLENPNKFDDEKYWITVDTYSAQGERATAFSNTLNNITSKYWRVVFDTKGDRYSSPVVPELQILGYPLPNADTIMKTVTTAKELSQQKDKFSQKMLDELKIKEMALETSLNSKIFDVTAINANAGVLKDCIEKRQLLKKGGGGSGGGGSGGGGSHHHHHHEFGGGGSGGGGSGGGGSAVTGTTKANIKLFSFTEVNDTNPLNNLNFTLKNSGKPLVDMVVLFSANINYDAANDKVFVSNNPNVQHLLTNRAKYLKPLQDKGIKVILSILGNHDRSGIANLSTARAKAFAQELKNTCDLYNLDGVFFDDEYSAYQTPPPSGFVTPSNNAAARLAYETKQAMPNKLVTVYVYSRTSSFPTAVDGVNAGSYVDYAIHDYGGSYDLATNYPGLAKSGMVMSSQEFNQGRYATAQALRNIVTKGYGGHMIFAMDPNRSNFTSGQLPALKLIAKELYGDELVYSNTPYSKDW

SEQ ID NO: 19 - protein, 600 aa, Artificial sequence
  EndoF3-EndoH
MATALAGSNGVCIAYYITDGRNPTFKLKDIPDKVDMVILFGLKYWSLQDTTKLPGGTGMMGSFKSYKDLDTQIRSLQSRGIKVLQNIDDDVSWQSSKPGGFASAAAYGDAIKSIVIDKWKLDGISLDIEHSGAKPNPIPTFPGYAATGYNGWYSGSMAATPAFLNVISELTKYFGTTAPNNKQLQIASGIDVYAWNKIMENFRNNFNYIQLQSYGANVSRTQLMMNYATGTNKIPASKMVFGAYAEGGTNQANDVEVAKWTPTQGAKGGMMIYTYNSNVSYANAVRDAVKNGGGGSGGGGSGGGGSHHHHHHEFGGGGSGGGGSGGGGSAPAPVKQGPTSVAYVEVNNNSMLNVGKYTLADGGGNAFDVAVIFAANINYDTGTKTAYLHFNENVQRVLDNAVTQIRPLQQQGIKVLLSVLGNHQGAGFANFPSQQAASAFAKQLSDAVAKYGLDGVDFDDEYAEYGNNGTAQPNDSSFVHLVTALRANMPDKIISLYNIGPAASRLSYGGVDVSDKFDYAWNPYYGTWQVPGIALPKAQLSPAAVEIGRTSRSTVADLARRTVDEGYGVYLTYNLDGGDRTADVSAFTRELYGSEAVRTP

SEQ ID NO: 20 - protein, 600 aa, Artificial sequence
  EndoF2-EndoH
MAVNLSNLIAYKNSDHQISAGYYRTWRDSATASGNLPSMRWLPDSLDMVMVFPDYTPPENAYWNTLKTNYVPYLHKRGTKVIITLGDLNSATTTGGQDSIGYSSWAKGIYDKWVGEYNLDGIDIDIESSPSGATLTKFVAATKALSKYFGPKSGTGKTFVYDTNQNPTNFFIQTAPRYNYVFLQAYGRSTTNLTTVSGLYAPYISMKQFLPGFSFYEENGYPGNYWNDVRYPQNGTGRAYDYARWQPATGKKGGVFSYAIERDAPLTSSNDNTLRAPNFRVTKDLIKIMNPGGGGSGGGGSGGGGSHHHHHHEFGGGGSGGGGSGGGGSAPAPVKQGPTSVAYVEVNNNSMLNVGKYTLADGGGNAFDVAVIFAANINYDTGTKTAYLHFNENVQRVLDNAVTQIRPLQQQGIKVLLSVLGNHQGAGFANFPSQQAASAFAKQLSDAVAKYGLDGVDFDDEYAEYGNNGTAQPNDSSFVHLVTALRANMPDKIISLYNIGPAASRLSYGGVDVSDKFDYAWNPYYGTWQVPGIALPKAQLSPAAVEIGRTSRSTVADLARRTVDEGYGVYLTYNLDGGDRTADVSAFTRELYGSEAVRTP

SEQ ID NO: 21 - protein, 1240 aa, Artificial sequence
  His6-EndoS-EndoH
MGSSHHHHHHSSGLVPRGSHMPSIDSLHYLSENSKKEFKEELSKAGQESQKVKEILAKAQQADKQAQELAKMKIPEKIPMKPLHGPLYGGYFRTWHDKTSDPTEKDKVNSMGELPKEVDLAFIFHDWTKDYSLFWKELATKHVPKLNKQGTRVIRTIPWRFLAGGDNSGIAEDTSKYPNTPEGNKALAKAIVDEYVYKYNLDGLDVDVEHDSIPKVDKKEDTAGVERSIQVFEEIGKLIGPKGVDKSRLFIMDSTYMADKNPLIERGAPYINLLLVQVYGSQGEKGGWEPVSNRPEKTMEERWQGYSKYIRPEQYMIGFSFYEENAQEGNLWYDINSRKDEDKANGINTDITGTRAERYARWQPKTGGVKGGIFSYAIDRDGVAHQPKKYAKQKEFKDATDNIFHSDYSVSKALKTVMLKDKSYDLIDEKDFPDKALREAVMAQVGTRKGDLERFNGTLRLDNPAIQSLEGLNKFKKLAQLDLIGLSRITKLDRSVLPANMKPGKDTLETVLETYKKDNKEEPATIPPVSLKVSGLTGLKELDLSGFDRETLAGLDAATLTSLEKVDISGNKLDLAPGTENRQIFDTMLSTISNHVGSNEQTVKFDKQKPTGHYPDTYGKTSLRLPVANEKVDLQSQLLFGTVTNQGTLINSEADYKAYQNHKIAGRSFVDSNYHYNNFKVSYENYTVKVTDSTLGTTTDKTLATDKEETYKVDFFSPADKTKAVHTAKVIVGDEKTMMVNLAEGATVIGGSADPVNARKVFDGQLGSETDNISLGWDSKQSIIFKLKEDGLIKHWRFFNDSARNPETTNKPIQEASLQIFNIKDYNLDNLLENPNKFDDEKYWITVDTYSAQGERATAFSNTLNNITSKYWRVVFDTKGDRYSSPVVPELQILGYPLPNADTIMKTVTTAKELSQQKDKFSQKMLDELKIKEMALETSLNSKIFDVTAINANAGVLKDCIEKRQLLKKAPAPVKQGPTSVAYVEVNNNSMLNVGKYTLADGGGNAFDVAVIFAANINYDTGTKTAYLHFNENVQRVLDNAVTQIRPLQQQGIKVLLSVLGNHQGAGFANFPSQQAASAFAKQLSDAVAKYGLDGVDFDDEYAEYGNNGTAQPNDSSFVHLVTALRANMPDKIISLYNIGPAASRLSYGGVDVSDKFDYAWNPYYGTWQVPGIALPKAQLSPAAVEIGRTSRSTVADLARRTVDEGYGVYLTYNLDGGDRTADVSAFTRELYGSEAVRTP

SEQ ID NO: 22 - DNA, 1812 bp, Artificial sequence
  synthetic DNA encoding fusion protein EndoF3-EfEndo18A
atggctacagcgctggctggttctaacggggtctgcatcgcgtattacatcaccgatgggcgtaatccgacgttcaaattgaaagacatcccggataaagtagacatggtaattctttttggtcttaagtattggtcattgcaggatacaaccaaattgccagggggtactggtatgatgggttcgtttaaatcctacaaggacctggacacccagattcgtagtcttcaaagccgtggaatcaaagtgttgcagaacattgacgacgacgtctcatggcagtcctcgaagccgggtgggttcgcttccgccgctgcttacggggatgctattaagagtatcgtaattgataagtggaagctggacgggattagcttggatattgagcattcgggggctaaacccaaccctatcccaacttttcctggatatgccgcgacaggatataatggctggtattcaggatctatggcagccacgcctgcctttcttaatgttatctcagagcttactaaatactttggtacaacggcaccgaataataagcaacttcagattgcttcgggtattgacgtatatgcctggaataaaatcatggagaactttcgtaataacttcaactacatccaattacagtcatacggagctaatgtctctcgtactcaacttatgatgaattacgcaacgggaactaataaaattcccgcctctaaaatggttttcggcgcctacgcagagggtggcactaaccaggcaaatgacgtggaggtcgccaagtggacacctacgcagggcgcaaagggcggtatgatgatctatacttacaattcgaacgtgagctatgcaaatgcggttcgcgacgcagtgaaaaatggcggcggcggctctggcggcggcggctctggcggcggcggctctcaccaccaccaccaccacgaattcggcggcggcggctctggcggcggcggctctggcggcggcggctctgcttcaaccgtaacccctaaaacggttatgtacgtagaagtaaataaccacgatttcaacaatgtcgggaaatacactcttgccggtactaatcagccggcgttcgatatgggtattatttttgccgccaacatcaattatgacaccgtcaataagaaaccatacctgtacttgaacgagcgcgtacagcaaacactgaatgaagcggagacgcagatccgtccggtccaggcacgtggaacgaaggttttgctttccatcttgggtaatcacgaaggcgcaggatttgccaattttcctacgtatgagtcggcggacgctttcgccgcgcaacttgagcaggttgtcaatacgtaccatttagacgggattgatttcgatgatgagtacgccgagtacggaaaaaacgggacccctcagccgaacaactcatccttcatctggttactgcaagctcttcgcaaccgtctgggaaatgataaacttatcactttctacaacattggcccggcagccgctaacagcagcgcaaaccctcaaatgtcatctttgattgactatgcctggaatccctattattcgacatggaaccccccacaaattgcaggtatgcctgcctcccgcctgggggcttctgcggttgaagtgggcgttaaccagaatcttgcagcacagtatgccaagcgtactaaggctgagcagtatggaatctatctgatgtacaatctgccaggaaaagattctagcgcttatatctcagcagcgactcaggagctgtatgggcgcaagacgaactatagccccacggtcccgactccgtgataa

SEQ ID NO: 23 - DNA, 1812 bp, Artificial sequence
  synthetic DNA encoding fusion protein EndoF2-EfEndo18A
atggcggtaaaccttagtaatcttatcgcttataaaaatagtgaccatcagatcagtgcgggatattaccgtacatggcgtgacagcgccacagccagtggtaatcttcctagtatgcgttggttgccagactcattggacatggtaatggtattcccagactatactcctccggaaaatgcgtattggaacacactgaagactaactacgtaccatacctgcataagcgtggcacgaaagttattatcacattgggggaccttaactctgcaacgaccacgggagggcaagattctattgggtattcatcgtgggccaaaggaatctatgataaatgggtgggcgagtataatcttgatggaatcgatattgacatcgaatcgtcaccgtccggtgcgaccttaacgaagtttgttgcggcaacaaaagcgttgtcaaagtattttggaccaaagagtgggacaggcaagacctttgtatacgataccaatcagaatccgactaatttctttatccaaactgccccacgctacaactacgtatttcttcaagcatacgggcgctcgaccactaatctgacgacggtctctggattatacgccccctatatttcaatgaaacaatttctgcccggcttctctttttacgaagaaaacggttacccaggtaattattggaatgatgtgcgttacccccagaacggtacaggccgtgcctacgactacgcgcgctggcagcccgccacgggaaaaaaaggaggggtgttcagttatgccatcgagcgcgacgcccctcttacatcgtcaaacgacaataccctgcgtgcgcctaactttcgtgtaacgaaggacttaatcaaaattatgaatcctggcggcggcggctctggcggcggcggctctggcggcggcggctctcaccaccaccaccaccacgaattcggcggcggcggctctggcggcggcggctctggcggcggcggctctgcttcaaccgtaacccctaaaacggttatgtacgtagaagtaaataaccacgatttcaacaatgtcgggaaatacactcttgccggtactaatcagccggcgttcgatatgggtattatttttgccgccaacatcaattatgacaccgtcaataagaaaccatacctgtacttgaacgagcgcgtacagcaaacactgaatgaagcggagacgcagatccgtccggtccaggcacgtggaacgaaggttttgctttccatcttgggtaatcacgaaggcgcaggatttgccaattttcctacgtatgagtcggcggacgctttcgccgcgcaacttgagcaggttgtcaatacgtaccatttagacgggattgatttcgatgatgagtacgccgagtacggaaaaaacgggacccctcagccgaacaactcatccttcatctggttactgcaagctcttcgcaaccgtctgggaaatgataaacttatcactttctacaacattggcccggcagccgctaacagcagcgcaaaccctcaaatgtcatctttgattgactatgcctggaatccctattattcgacatggaaccccccacaaattgcaggtatgcctgcctcccgcctgggggcttctgcggttgaagtgggcgttaaccagaatcttgcagcacagtatgccaagcgtactaaggctgagcagtatggaatctatctgatgtacaatctgccaggaaaagattctagcgcttatatctcagcagcgactcaggagctgtatgggcgcaagacgaactatagccccacggtcccgactccgtgataa

SEQ ID NO: 24 - DNA, 3786 bp, Artificial sequence
  synthetic DNA encoding fusion protein EndoS-EfEndo18A
atgccgtcaatcgattcgctgcattatctgagcgaaaactctaaaaaagaatttaaagaagaactgagcaaagcgggccaggaatctcaaaaagttaaagaaatcctggcaaaagctcagcaagccgataaacaggcacaagaactggctaaaatgaaaattccggaaaaaatcccgatgaaaccgctgcatggtccgctgtacggcggttatttccgtacctggcacgataaaacgtcagacccgaccgaaaaagacaaagtcaactcgatgggcgaactgccgaaagaagtggatctggcttttattttccatgattggaccaaagactactctctgttttggaaagaactggcaacgaaacacgttccgaaactgaacaaacagggtacgcgtgtcattcgtaccattccgtggcgcttcctggctggcggtgataattcaggcatcgcggaagacacctcgaaatatccgaacacgccggaaggtaataaagcgctggccaaagcaatcgtcgatgaatacgtgtacaaatacaatctggacggcctggatgtggacgttgaacatgattcaattccgaaagtggataaaaaagaagacaccgccggcgtggaacgttcgatccaggtttttgaagaaattggtaaactgatcggcccgaaaggtgttgataaaagccgtctgttcatcatggattctacctatatggccgacaaaaatccgctgattgaacgcggtgcaccgtacatcaacctgctgctggtccaggtgtatggcagccaaggtgaaaaaggcggttgggaaccggtgtctaaccgtccggaaaaaaccatggaagaacgctggcagggctactcaaaatatattcgtccggaacaatacatgatcggcttttcgttctatgaagaaaacgcgcaggaaggtaatctgtggtacgatattaatagtcgcaaagatgaagacaaagccaacggcattaataccgatatcacgggtacccgtgcggaacgctatgcccgttggcagccgaaaaccggcggtgttaaaggcggtatttttagctacgcgatcgatcgtgacggtgtcgcccatcagccgaaaaaatacgcaaaacaaaaagagttcaaagatgctaccgacaacatcttccacagcgattacagtgtctccaaagcgctgaaaaccgtgatgctgaaagataaatcttacgatctgatcgacgaaaaagattttccggacaaagcgctgcgcgaagccgttatggcacaggtcggcacccgcaaaggtgacctggaacgttttaatggcacgctgcgcctggataacccggccattcagagcctggaaggtctgaataaattcaaaaaactggcacaactggacctgattggcctgagccgtatcaccaaactggatcgctctgtgctgccggccaacatgaaaccgggtaaagacacgctggaaaccgttctggaaacctacaaaaaagataacaaagaagaaccggcaacgatcccgccggtgtctctgaaagtttccggcctgaccggtctgaaagaactggatctgagcggctttgaccgtgaaacgctggcaggtctggatgcggccacgctgaccagtctggaaaaagttgatatttccggcaataaactggacctggcgccgggtaccgaaaaccgccagatttttgatacgatgctgagtaccatctccaaccatgttggcagcaatgaacagaccgtcaaattcgacaaacaaaaaccgacgggccactacccggatacgtatggtaaaaccagcctgcgtctgccggtcgccaacgaaaaagtggatctgcagtctcaactgctgtttggcacggttaccaatcagggtaccctgattaacagcgaagcagattacaaggcttaccaaaaccataaaatcgcgggtcgctcatttgtggattcgaactaccactacaacaacttcaaagttagttacgaaaactacaccgttaaagtcacggattccaccctgggcaccacgaccgataaaacgctggccaccgacaaagaagaaacctacaaagtcgatttctttagcccggcagacaaaacgaaagcggtgcataccgccaaagtgattgttggcgatgaaaaaaccatgatggtgaacctggctgaaggtgcgacggttatcggcggttccgcagacccggttaacgctcgcaaagtctttgatggccagctgggtagtgaaaccgataatatttccctgggttgggactcaaaacagtcgattatcttcaaactgaaagaagacggcctgatcaaacactggcgtttctttaacgatagtgcccgcaatccggaaacgaccaacaaaccgattcaggaagcatccctgcaaatcttcaacatcaaagattacaacctggacaatctgctggaaaacccgaataaattcgatgacgaaaaatactggatcacggtggatacctatagcgcgcagggcgaacgtgctacggcgtttagtaacaccctgaacaatattacgtccaaatactggcgtgtggttttcgataccaaaggtgaccgctatagctctccggtcgtgccggaactgcagattctgggctatccgctgccgaatgctgatacgatcatgaaaaccgtgacgaccgcgaaagaactgtcacagcaaaaagataaattctcgcagaaaatgctggacgaactgaaaattaaagaaatggctctggaaaccagcctgaacagtaaaattttcgatgttacggcgatcaatgctaacgctggtgtgctgaaagactgtattgaaaaacgccaactgctgaaaaaaggcggcggcggctctggcggcggcggctctggcggcggcggctctcaccaccaccaccaccacgaattcggcggcggcggctctggcggcggcggctctggcggcggcggctctgcttcaaccgtaacccctaaaacggttatgtacgtagaagtaaataaccacgatttcaacaatgtcgggaaatacactcttgccggtactaatcagccggcgttcgatatgggtattatttttgccgccaacatcaattatgacaccgtcaataagaaaccatacctgtacttgaacgagcgcgtacagcaaacactgaatgaagcggagacgcagatccgtccggtccaggcacgtggaacgaaggttttgctttccatcttgggtaatcacgaaggcgcaggatttgccaattttcctacgtatgagtcggcggacgctttcgccgcgcaacttgagcaggttgtcaatacgtaccatttagacgggattgatttcgatgatgagtacgccgagtacggaaaaaacgggacccctcagccgaacaactcatccttcatctggttactgcaagctcttcgcaaccgtctgggaaatgataaacttatcactttctacaacattggcccggcagccgctaacagcagcgcaaaccctcaaatgtcatctttgattgactatgcctggaatccctattattcgacatggaaccccccacaaattgcaggtatgcctgcctcccgcctgggggcttctgcggttgaagtgggcgttaaccagaatcttgcagcacagtatgccaagcgtactaaggctgagcagtatggaatctatctgatgtacaatctgccaggaaaagattctagcgcttatatctcagcagcgactcaggagctgtatgggcgcaagacgaactatagccccacggtcccgactccgtgataa

SEQ ID NO: 25 - DNA, 1860 bp, Artificial sequence
  synthetic DNA encoding fusion protein EndoF3-EndoF1
atggctacagcgctggctggttctaacggggtctgcatcgcgtattacatcaccgatgggcgtaatccgacgttcaaattgaaagacatcccggataaagtagacatggtaattctttttggtcttaagtattggtcattgcaggatacaaccaaattgccagggggtactggtatgatgggttcgtttaaatcctacaaggacctggacacccagattcgtagtcttcaaagccgtggaatcaaagtgttgcagaacattgacgacgacgtctcatggcagtcctcgaagccgggtgggttcgcttccgccgctgcttacggggatgctattaagagtatcgtaattgataagtggaagctggacgggattagcttggatattgagcattcgggggctaaacccaaccctatcccaacttttcctggatatgccgcgacaggatataatggctggtattcaggatctatggcagccacgcctgcctttcttaatgttatctcagagcttactaaatactttggtacaacggcaccgaataataagcaacttcagattgcttcgggtattgacgtatatgcctggaataaaatcatggagaactttcgtaataacttcaactacatccaattacagtcatacggagctaatgtctctcgtactcaacttatgatgaattacgcaacgggaactaataaaattcccgcctctaaaatggttttcggcgcctacgcagagggtggcactaaccaggcaaatgacgtggaggtcgccaagtggacacctacgcagggcgcaaagggcggtatgatgatctatacttacaattcgaacgtgagctatgcaaatgcggttcgcgacgcagtgaaaaatggcggcggcggctctggcggcggcggctctggcggcggcggctctcaccaccaccaccaccacgaattcggcggcggcggctctggcggcggcggctctggcggcggcggctctgcggtaaccgggacaacgaaggctaacatcaaactttttagttttacagaggtaaacgacactaatccgttgaacaatctgaactttaccttaaaaaactcgggaaaacccttagtagatatggtagtgttattttccgcgaacattaactatgacgcggccaacgataaggtcttcgtatcgaataatccgaacgtacagcatcttttgaccaatcgtgcgaagtaccttaagccgttacaagacaaggggatcaaggtgattttgtcaatcttagggaaccatgatcgctccgggatcgccaatttgagtacggctcgtgcgaaggcatttgctcaggaactgaagaatacttgcgatttgtataatttagacggggtattctttgatgatgagtactctgcttaccaaacgccaccgccgagcggcttcgtgacacccagtaataacgccgcagctcgccttgcttatgaaacaaagcaggctatgccaaacaagctggtcacggtgtacgtctattcccgcacttcgagttttcccacagcggtagacggggtcaacgccgggtcctacgtagactatgcgattcatgactacggtggctcatacgacttggctactaattatccggggttggctaagtctgggatggtgatgtctagtcaggagtttaaccagggccgttacgcgactgcacaagcattgcgcaacattgtgaccaagggctatggaggccacatgatctttgccatggaccccaatcgttctaatttcacgtcagggcaactgcccgcactgaagctgattgccaaggagctttacggggatgagcttgtgtacagcaacactccttacagtaaggattggtgataa

SEQ ID NO: 26 - DNA, 1860 bp, Artificial sequence
  DNA encoding fusion protein EndoF2-EndoF1
atggcggtaaaccttagtaatcttatcgcttataaaaatagtgaccatcagatcagtgcgggatattaccgtacatggcgtgacagcgccacagccagtggtaatcttcctagtatgcgttggttgccagactcattggacatggtaatggtattcccagactatactcctccggaaaatgcgtattggaacacactgaagactaactacgtaccatacctgcataagcgtggcacgaaagttattatcacattgggggaccttaactctgcaacgaccacgggagggcaagattctattgggtattcatcgtgggccaaaggaatctatgataaatgggtgggcgagtataatcttgatggaatcgatattgacatcgaatcgtcaccgtccggtgcgaccttaacgaagtttgttgcggcaacaaaagcgttgtcaaagtattttggaccaaagagtgggacaggcaagacctttgtatacgataccaatcagaatccgactaatttctttatccaaactgccccacgctacaactacgtatttcttcaagcatacgggcgctcgaccactaatctgacgacggtctctggattatacgccccctatatttcaatgaaacaatttctgcccggcttctctttttacgaagaaaacggttacccaggtaattattggaatgatgtgcgttacccccagaacggtacaggccgtgcctacgactacgcgcgctggcagcccgccacgggaaaaaaaggaggggtgttcagttatgccatcgagcgcgacgcccctcttacatcgtcaaacgacaataccctgcgtgcgcctaactttcgtgtaacgaaggacttaatcaaaattatgaatcctggcggcggcggctctggcggcggcggctctggcggcggcggctctcaccaccaccaccaccacgaattcggcggcggcggctctggcggcggcggctctggcggcggcggctctgcggtaaccgggacaacgaaggctaacatcaaactttttagttttacagaggtaaacgacactaatccgttgaacaatctgaactttaccttaaaaaactcgggaaaacccttagtagatatggtagtgttattttccgcgaacattaactatgacgcggccaacgataaggtcttcgtatcgaataatccgaacgtacagcatcttttgaccaatcgtgcgaagtaccttaagccgttacaagacaaggggatcaaggtgattttgtcaatcttagggaaccatgatcgctccgggatcgccaatttgagtacggctcgtgcgaaggcatttgctcaggaactgaagaatacttgcgatttgtataatttagacggggtattctttgatgatgagtactctgcttaccaaacgccaccgccgagcggcttcgtgacacccagtaataacgccgcagctcgccttgcttatgaaacaaagcaggctatgccaaacaagctggtcacggtgtacgtctattcccgcacttcgagttttcccacagcggtagacggggtcaacgccgggtcctacgtagactatgcgattcatgactacggtggctcatacgacttggctactaattatccggggttggctaagtctgggatggtgatgtctagtcaggagtttaaccagggccgttacgcgactgcacaagcattgcgcaacattgtgaccaagggctatggaggccacatgatctttgccatggaccccaatcgttctaatttcacgtcagggcaactgcccgcactgaagctgattgccaaggagctttacggggatgagcttgtgtacagcaacactccttacagtaaggattggtgataa

SEQ ID NO: 27 - DNA, 3834 bp, Artificial sequence
  synthetic DNA encoding fusion protein EndoS-EndoF1
atgccgtcaatcgattcgctgcattatctgagcgaaaactctaaaaaagaatttaaagaagaactgagcaaagcgggccaggaatctcaaaaagttaaagaaatcctggcaaaagctcagcaagccgataaacaggcacaagaactggctaaaatgaaaattccggaaaaaatcccgatgaaaccgctgcatggtccgctgtacggcggttatttccgtacctggcacgataaaacgtcagacccgaccgaaaaagacaaagtcaactcgatgggcgaactgccgaaagaagtggatctggcttttattttccatgattggaccaaagactactctctgttttggaaagaactggcaacgaaacacgttccgaaactgaacaaacagggtacgcgtgtcattcgtaccattccgtggcgcttcctggctggcggtgataattcaggcatcgcggaagacacctcgaaatatccgaacacgccggaaggtaataaagcgctggccaaagcaatcgtcgatgaatacgtgtacaaatacaatctggacggcctggatgtggacgttgaacatgattcaattccgaaagtggataaaaaagaagacaccgccggcgtggaacgttcgatccaggtttttgaagaaattggtaaactgatcggcccgaaaggtgttgataaaagccgtctgttcatcatggattctacctatatggccgacaaaaatccgctgattgaacgcggtgcaccgtacatcaacctgctgctggtccaggtgtatggcagccaaggtgaaaaaggcggttgggaaccggtgtctaaccgtccggaaaaaaccatggaagaacgctggcagggctactcaaaatatattcgtccggaacaatacatgatcggcttttcgttctatgaagaaaacgcgcaggaaggtaatctgtggtacgatattaatagtcgcaaagatgaagacaaagccaacggcattaataccgatatcacgggtacccgtgcggaacgctatgcccgttggcagccgaaaaccggcggtgttaaaggcggtatttttagctacgcgatcgatcgtgacggtgtcgcccatcagccgaaaaaatacgcaaaacaaaaagagttcaaagatgctaccgacaacatcttccacagcgattacagtgtctccaaagcgctgaaaaccgtgatgctgaaagataaatcttacgatctgatcgacgaaaaagattttccggacaaagcgctgcgcgaagccgttatggcacaggtcggcacccgcaaaggtgacctggaacgttttaatggcacgctgcgcctggataacccggccattcagagcctggaaggtctgaataaattcaaaaaactggcacaactggacctgattggcctgagccgtatcaccaaactggatcgctctgtgctgccggccaacatgaaaccgggtaaagacacgctggaaaccgttctggaaacctacaaaaaagataacaaagaagaaccggcaacgatcccgccggtgtctctgaaagtttccggcctgaccggtctgaaagaactggatctgagcggctttgaccgtgaaacgctggcaggtctggatgcggccacgctgaccagtctggaaaaagttgatatttccggcaataaactggacctggcgccgggtaccgaaaaccgccagatttttgatacgatgctgagtaccatctccaaccatgttggcagcaatgaacagaccgtcaaattcgacaaacaaaaaccgacgggccactacccggatacgtatggtaaaaccagcctgcgtctgccggtcgccaacgaaaaagtggatctgcagtctcaactgctgtttggcacggttaccaatcagggtaccctgattaacagcgaagcagattacaaggcttaccaaaaccataaaatcgcgggtcgctcatttgtggattcgaactaccactacaacaacttcaaagttagttacgaaaactacaccgttaaagtcacggattccaccctgggcaccacgaccgataaaacgctggccaccgacaaagaagaaacctacaaagtcgatttctttagcccggcagacaaaacgaaagcggtgcataccgccaaagtgattgttggcgatgaaaaaaccatgatggtgaacctggctgaaggtgcgacggttatcggcggttccgcagacccggttaacgctcgcaaagtctttgatggccagctgggtagtgaaaccgataatatttccctgggttgggactcaaaacagtcgattatcttcaaactgaaagaagacggcctgatcaaacactggcgtttctttaacgatagtgcccgcaatccggaaacgaccaacaaaccgattcaggaagcatccctgcaaatcttcaacatcaaagattacaacctggacaatctgctggaaaacccgaataaattcgatgacgaaaaatactggatcacggtggatacctatagcgcgcagggcgaacgtgctacggcgtttagtaacaccctgaacaatattacgtccaaatactggcgtgtggttttcgataccaaaggtgaccgctatagctctccggtcgtgccggaactgcagattctgggctatccgctgccgaatgctgatacgatcatgaaaaccgtgacgaccgcgaaagaactgtcacagcaaaaagataaattctcgcagaaaatgctggacgaactgaaaattaaagaaatggctctggaaaccagcctgaacagtaaaattttcgatgttacggcgatcaatgctaacgctggtgtgctgaaagactgtattgaaaaacgccaactgctgaaaaaaggcggcggcggctctggcggcggcggctctggcggcggcggctctcaccaccaccaccaccacgaattcggcggcggcggctctggcggcggcggctctggcggcggcggctctgcggtaaccgggacaacgaaggctaacatcaaactttttagttttacagaggtaaacgacactaatccgttgaacaatctgaactttaccttaaaaaactcgggaaaacccttagtagatatggtagtgttattttccgcgaacattaactatgacgcggccaacgataaggtcttcgtatcgaataatccgaacgtacagcatcttttgaccaatcgtgcgaagtaccttaagccgttacaagacaaggggatcaaggtgattttgtcaatcttagggaaccatgatcgctccgggatcgccaatttgagtacggctcgtgcgaaggcatttgctcaggaactgaagaatacttgcgatttgtataatttagacggggtattctttgatgatgagtactctgcttaccaaacgccaccgccgagcggcttcgtgacacccagtaataacgccgcagctcgccttgcttatgaaacaaagcaggctatgccaaacaagctggtcacggtgtacgtctattcccgcacttcgagttttcccacagcggtagacggggtcaacgccgggtcctacgtagactatgcgattcatgactacggtggctcatacgacttggctactaattatccggggttggctaagtctgggatggtgatgtctagtcaggagtttaaccagggccgttacgcgactgcacaagcattgcgcaacattgtgaccaagggctatggaggccacatgatctttgccatggaccccaatcgttctaatttcacgtcagggcaactgcccgcactgaagctgattgccaaggagctttacggggatgagcttgtgtacagcaacactccttacagtaaggattggtgataa

SEQ ID NO: 28 - DNA, 1806 bp, Artificial sequence
  synthetic DNA encoding fusion protein EndoF3-EndoH
atggctacagcgctggctggttctaacggggtctgcatcgcgtattacatcaccgatgggcgtaatccgacgttcaaattgaaagacatcccggataaagtagacatggtaattctttttggtcttaagtattggtcattgcaggatacaaccaaattgccagggggtactggtatgatgggttcgtttaaatcctacaaggacctggacacccagattcgtagtcttcaaagccgtggaatcaaagtgttgcagaacattgacgacgacgtctcatggcagtcctcgaagccgggtgggttcgcttccgccgctgcttacggggatgctattaagagtatcgtaattgataagtggaagctggacgggattagcttggatattgagcattcgggggctaaacccaaccctatcccaacttttcctggatatgccgcgacaggatataatggctggtattcaggatctatggcagccacgcctgcctttcttaatgttatctcagagcttactaaatactttggtacaacggcaccgaataataagcaacttcagattgcttcgggtattgacgtatatgcctggaataaaatcatggagaactttcgtaataacttcaactacatccaattacagtcatacggagctaatgtctctcgtactcaacttatgatgaattacgcaacgggaactaataaaattcccgcctctaaaatggttttcggcgcctacgcagagggtggcactaaccaggcaaatgacgtggaggtcgccaagtggacacctacgcagggcgcaaagggcggtatgatgatctatacttacaattcgaacgtgagctatgcaaatgcggttcgcgacgcagtgaaaaatggcggcggcggctctggcggcggcggctctggcggcggcggctctcaccaccaccaccaccacgaattcggcggcggcggctctggcggcggcggctctggcggcggcggctctgccccggccccggtgaagcaggggccgacctcggtggcctacgtcgaggtgaacaacaacagcatgctcaacgtcggcaagtacaccctggcggacggaggcggcaacgccttcgacgtagccgtgatcttcgcggcgaacatcaactacgacaccggcacgaagacggcctacctgcacttcaacgagaacgtgcagcgcgtccttgacaacgctgtcacgcagatacggccgttgcagcaacagggcatcaaggtcctcctctcggtgctcggcaaccaccagggcgccgggttcgcgaacttcccctcacagcaggcggcttcggcgttcgcgaagcagctctcggacgccgtggcgaagtacggcctcgacggcgtcgacttcgacgacgaatacgccgagtacggcaacaacggcaccgcgcagcccaacgacagttcgttcgtgcacctggtgacggcactgcgcgcgaacatgcccgacaagatcatcagcctctacaacatcggcccggccgcgtcccgcctgtcgtacggcggtgtcgacgtctccgacaagttcgactacgcctggaatccctactacggcacctggcaggtccccggcatcgcactgcccaaggcgcagctgtcgccggcggccgtcgagatcggccggacctcacggagcaccgtcgccgacctcgcccgtcgcaccgtcgacgaggggtacggcgtctatctgacgtacaacctcgacggcggcgatcgcaccgccgacgtctccgcgttcaccagggagctgtacggcagcgaggcggtccggacgccgtgataa

SEQ ID NO: 29 - DNA, 1806 bp, Artificial sequence
  synthetic DNA encoding fusion protein EndoF2-EndoH
atggcggtaaaccttagtaatcttatcgcttataaaaatagtgaccatcagatcagtgcgggatattaccgtacatggcgtgacagcgccacagccagtggtaatcttcctagtatgcgttggttgccagactcattggacatggtaatggtattcccagactatactcctccggaaaatgcgtattggaacacactgaagactaactacgtaccatacctgcataagcgtggcacgaaagttattatcacattgggggaccttaactctgcaacgaccacgggagggcaagattctattgggtattcatcgtgggccaaaggaatctatgataaatgggtgggcgagtataatcttgatggaatcgatattgacatcgaatcgtcaccgtccggtgcgaccttaacgaagtttgttgcggcaacaaaagcgttgtcaaagtattttggaccaaagagtgggacaggcaagacctttgtatacgataccaatcagaatccgactaatttctttatccaaactgccccacgctacaactacgtatttcttcaagcatacgggcgctcgaccactaatctgacgacggtctctggattatacgccccctatatttcaatgaaacaatttctgcccggcttctctttttacgaagaaaacggttacccaggtaattattggaatgatgtgcgttacccccagaacggtacaggccgtgcctacgactacgcgcgctggcagcccgccacgggaaaaaaaggaggggtgttcagttatgccatcgagcgcgacgcccctcttacatcgtcaaacgacaataccctgcgtgcgcctaactttcgtgtaacgaaggacttaatcaaaattatgaatcctggcggcggcggctctggcggcggcggctctggcggcggcggctctcaccaccaccaccaccacgaattcggcggcggcggctctggcggcggcggctctggcggcggcggctctgccccggccccggtgaagcaggggccgacctcggtggcctacgtcgaggtgaacaacaacagcatgctcaacgtcggcaagtacaccctggcggacggaggcggcaacgccttcgacgtagccgtgatcttcgcggcgaacatcaactacgacaccggcacgaagacggcctacctgcacttcaacgagaacgtgcagcgcgtccttgacaacgctgtcacgcagatacggccgttgcagcaacagggcatcaaggtcctcctctcggtgctcggcaaccaccagggcgccgggttcgcgaacttcccctcacagcaggcggcttcggcgttcgcgaagcagctctcggacgccgtggcgaagtacggcctcgacggcgtcgacttcgacgacgaatacgccgagtacggcaacaacggcaccgcgcagcccaacgacagttcgttcgtgcacctggtgacggcactgcgcgcgaacatgcccgacaagatcatcagcctctacaacatcggcccggccgcgtcccgcctgtcgtacggcggtgtcgacgtctccgacaagttcgactacgcctggaatccctactacggcacctggcaggtccccggcatcgcactgcccaaggcgcagctgtcgccggcggccgtcgagatcggccggacctcacggagcaccgtcgccgacctcgcccgtcgcaccgtcgacgaggggtacggcgtctatctgacgtacaacctcgacggcggcgatcgcaccgccgacgtctccgcgttcaccagggagctgtacggcagcgaggcggtccggacgccgtgataa

SEQ ID NO: 30 - DNA, 3780 bp, Artificial sequence
  synthetic DNA encoding fusion protein EndoS-EndoH (or EndoSH)
atgccgtcaatcgattcgctgcattatctgagcgaaaactctaaaaaagaatttaaagaagaactgagcaaagcgggccaggaatctcaaaaagttaaagaaatcctggcaaaagctcagcaagccgataaacaggcacaagaactggctaaaatgaaaattccggaaaaaatcccgatgaaaccgctgcatggtccgctgtacggcggttatttccgtacctggcacgataaaacgtcagacccgaccgaaaaagacaaagtcaactcgatgggcgaactgccgaaagaagtggatctggcttttattttccatgattggaccaaagactactctctgttttggaaagaactggcaacgaaacacgttccgaaactgaacaaacagggtacgcgtgtcattcgtaccattccgtggcgcttcctggctggcggtgataattcaggcatcgcggaagacacctcgaaatatccgaacacgccggaaggtaataaagcgctggccaaagcaatcgtcgatgaatacgtgtacaaatacaatctggacggcctggatgtggacgttgaacatgattcaattccgaaagtggataaaaaagaagacaccgccggcgtggaacgttcgatccaggtttttgaagaaattggtaaactgatcggcccgaaaggtgttgataaaagccgtctgttcatcatggattctacctatatggccgacaaaaatccgctgattgaacgcggtgcaccgtacatcaacctgctgctggtccaggtgtatggcagccaaggtgaaaaaggcggttgggaaccggtgtctaaccgtccggaaaaaaccatggaagaacgctggcagggctactcaaaatatattcgtccggaacaatacatgatcggcttttcgttctatgaagaaaacgcgcaggaaggtaatctgtggtacgatattaatagtcgcaaagatgaagacaaagccaacggcattaataccgatatcacgggtacccgtgcggaacgctatgcccgttggcagccgaaaaccggcggtgttaaaggcggtatttttagctacgcgatcgatcgtgacggtgtcgcccatcagccgaaaaaatacgcaaaacaaaaagagttcaaagatgctaccgacaacatcttccacagcgattacagtgtctccaaagcgctgaaaaccgtgatgctgaaagataaatcttacgatctgatcgacgaaaaagattttccggacaaagcgctgcgcgaagccgttatggcacaggtcggcacccgcaaaggtgacctggaacgttttaatggcacgctgcgcctggataacccggccattcagagcctggaaggtctgaataaattcaaaaaactggcacaactggacctgattggcctgagccgtatcaccaaactggatcgctctgtgctgccggccaacatgaaaccgggtaaagacacgctggaaaccgttctggaaacctacaaaaaagataacaaagaagaaccggcaacgatcccgccggtgtctctgaaagtttccggcctgaccggtctgaaagaactggatctgagcggctttgaccgtgaaacgctggcaggtctggatgcggccacgctgaccagtctggaaaaagttgatatttccggcaataaactggacctggcgccgggtaccgaaaaccgccagatttttgatacgatgctgagtaccatctccaaccatgttggcagcaatgaacagaccgtcaaattcgacaaacaaaaaccgacgggccactacccggatacgtatggtaaaaccagcctgcgtctgccggtcgccaacgaaaaagtggatctgcagtctcaactgctgtttggcacggttaccaatcagggtaccctgattaacagcgaagcagattacaaggcttaccaaaaccataaaatcgcgggtcgctcatttgtggattcgaactaccactacaacaacttcaaagttagttacgaaaactacaccgttaaagtcacggattccaccctgggcaccacgaccgataaaacgctggccaccgacaaagaagaaacctacaaagtcgatttctttagcccggcagacaaaacgaaagcggtgcataccgccaaagtgattgttggcgatgaaaaaaccatgatggtgaacctggctgaaggtgcgacggttatcggcggttccgcagacccggttaacgctcgcaaagtctttgatggccagctgggtagtgaaaccgataatatttccctgggttgggactcaaaacagtcgattatcttcaaactgaaagaagacggcctgatcaaacactggcgtttctttaacgatagtgcccgcaatccggaaacgaccaacaaaccgattcaggaagcatccctgcaaatcttcaacatcaaagattacaacctggacaatctgctggaaaacccgaataaattcgatgacgaaaaatactggatcacggtggatacctatagcgcgcagggcgaacgtgctacggcgtttagtaacaccctgaacaatattacgtccaaatactggcgtgtggttttcgataccaaaggtgaccgctatagctctccggtcgtgccggaactgcagattctgggctatccgctgccgaatgctgatacgatcatgaaaaccgtgacgaccgcgaaagaactgtcacagcaaaaagataaattctcgcagaaaatgctggacgaactgaaaattaaagaaatggctctggaaaccagcctgaacagtaaaattttcgatgttacggcgatcaatgctaacgctggtgtgctgaaagactgtattgaaaaacgccaactgctgaaaaaaggcggcggcggctctggcggcggcggctctggcggcggcggctctcaccaccaccaccaccacgaattcggcggcggcggctctggcggcggcggctctggcggcggcggctctgccccggccccggtgaagcaggggccgacctcggtggcctacgtcgaggtgaacaacaacagcatgctcaacgtcggcaagtacaccctggcggacggaggcggcaacgccttcgacgtagccgtgatcttcgcggcgaacatcaactacgacaccggcacgaagacggcctacctgcacttcaacgagaacgtgcagcgcgtccttgacaacgctgtcacgcagatacggccgttgcagcaacagggcatcaaggtcctcctctcggtgctcggcaaccaccagggcgccgggttcgcgaacttcccctcacagcaggcggcttcggcgttcgcgaagcagctctcggacgccgtggcgaagtacggcctcgacggcgtcgacttcgacgacgaatacgccgagtacggcaacaacggcaccgcgcagcccaacgacagttcgttcgtgcacctggtgacggcactgcgcgcgaacatgcccgacaagatcatcagcctctacaacatcggcccggccgcgtcccgcctgtcgtacggcggtgtcgacgtctccgacaagttcgactacgcctggaatccctactacggcacctggcaggtccccggcatcgcactgcccaaggcgcagctgtcgccggcggccgtcgagatcggccggacctcacggagcaccgtcgccgacctcgcccgtcgcaccgtcgacgaggggtacggcgtctatctgacgtacaacctcgacggcggcgatcgcaccgccgacgtctccgcgttcaccagggagctgtacggcagcgaggcggtccggacgccgtgataa

SEQ ID NO: 31 - DNA, 3726 bp, Artificial sequence
  synthetic DNA encoding fusion protein His6-EndoS-EndoH (EndoS-EndoH without GS-linker)
atgggcagcagccatcatcatcatcatcacagcagcggcctggtgccgcgcggcagccatatgccgtcaatcgattcgctgcattatctgagcgaaaactctaaaaaagaatttaaagaagaactgagcaaagcgggccaggaatctcaaaaagttaaagaaatcctggcaaaagctcagcaagccgataaacaggcacaagaactggctaaaatgaaaattccggaaaaaatcccgatgaaaccgctgcatggtccgctgtacggcggttatttccgtacctggcacgataaaacgtcagacccgaccgaaaaagacaaagtcaactcgatgggcgaactgccgaaagaagtggatctggcttttattttccatgattggaccaaagactactctctgttttggaaagaactggcaacgaaacacgttccgaaactgaacaaacagggtacgcgtgtcattcgtaccattccgtggcgcttcctggctggcggtgataattcaggcatcgcggaagacacctcgaaatatccgaacacgccggaaggtaataaagcgctggccaaagcaatcgtcgatgaatacgtgtacaaatacaatctggacggcctggatgtggacgttgaacatgattcaattccgaaagtggataaaaaagaagacaccgccggcgtggaacgttcgatccaggtttttgaagaaattggtaaactgatcggcccgaaaggtgttgataaaagccgtctgttcatcatggattctacctatatggccgacaaaaatccgctgattgaacgcggtgcaccgtacatcaacctgctgctggtccaggtgtatggcagccaaggtgaaaaaggcggttgggaaccggtgtctaaccgtccggaaaaaaccatggaagaacgctggcagggctactcaaaatatattcgtccggaacaatacatgatcggcttttcgttctatgaagaaaacgcgcaggaaggtaatctgtggtacgatattaatagtcgcaaagatgaagacaaagccaacggcattaataccgatatcacgggtacccgtgcggaacgctatgcccgttggcagccgaaaaccggcggtgttaaaggcggtatttttagctacgcgatcgatcgtgacggtgtcgcccatcagccgaaaaaatacgcaaaacaaaaagagttcaaagatgctaccgacaacatcttccacagcgattacagtgtctccaaagcgctgaaaaccgtgatgctgaaagataaatcttacgatctgatcgacgaaaaagattttccggacaaagcgctgcgcgaagccgttatggcacaggtcggcacccgcaaaggtgacctggaacgttttaatggcacgctgcgcctggataacccggccattcagagcctggaaggtctgaataaattcaaaaaactggcacaactggacctgattggcctgagccgtatcaccaaactggatcgctctgtgctgccggccaacatgaaaccgggtaaagacacgctggaaaccgttctggaaacctacaaaaaagataacaaagaagaaccggcaacgatcccgccggtgtctctgaaagtttccggcctgaccggtctgaaagaactggatctgagcggctttgaccgtgaaacgctggcaggtctggatgcggccacgctgaccagtctggaaaaagttgatatttccggcaataaactggacctggcgccgggtaccgaaaaccgccagatttttgatacgatgctgagtaccatctccaaccatgttggcagcaatgaacagaccgtcaaattcgacaaacaaaaaccgacgggccactacccggatacgtatggtaaaaccagcctgcgtctgccggtcgccaacgaaaaagtggatctgcagtctcaactgctgtttggcacggttaccaatcagggtaccctgattaacagcgaagcagattacaaggcttaccaaaaccataaaatcgcgggtcgctcatttgtggattcgaactaccactacaacaacttcaaagttagttacgaaaactacaccgttaaagtcacggattccaccctgggcaccacgaccgataaaacgctggccaccgacaaagaagaaacctacaaagtcgatttctttagcccggcagacaaaacgaaagcggtgcataccgccaaagtgattgttggcgatgaaaaaaccatgatggtgaacctggctgaaggtgcgacggttatcggcggttccgcagacccggttaacgctcgcaaagtctttgatggccagctgggtagtgaaaccgataatatttccctgggttgggactcaaaacagtcgattatcttcaaactgaaagaagacggcctgatcaaacactggcgtttctttaacgatagtgcccgcaatccggaaacgaccaacaaaccgattcaggaagcatccctgcaaatcttcaacatcaaagattacaacctggacaatctgctggaaaacccgaataaattcgatgacgaaaaatactggatcacggtggatacctatagcgcgcagggcgaacgtgctacggcgtttagtaacaccctgaacaatattacgtccaaatactggcgtgtggttttcgataccaaaggtgaccgctatagctctccggtcgtgccggaactgcagattctgggctatccgctgccgaatgctgatacgatcatgaaaaccgtgacgaccgcgaaagaactgtcacagcaaaaagataaattctcgcagaaaatgctggacgaactgaaaattaaagaaatggctctggaaaccagcctgaacagtaaaattttcgatgttacggcgatcaatgctaacgctggtgtgctgaaagactgtattgaaaaacgccaactgctgaaaaaagccccggccccggtgaagcaggggccgacctcggtggcctacgtcgaggtgaacaacaacagcatgctcaacgtcggcaagtacaccctggcggacggaggcggcaacgccttcgacgtagccgtgatcttcgcggcgaacatcaactacgacaccggcacgaagacggcctacctgcacttcaacgagaacgtgcagcgcgtccttgacaacgctgtcacgcagatacggccgttgcagcaacagggcatcaaggtcctcctctcggtgctcggcaaccaccagggcgccgggttcgcgaacttcccctcacagcaggcggcttcggcgttcgcgaagcagctctcggacgccgtggcgaagtacggcctcgacggcgtcgacttcgacgacgaatacgccgagtacggcaacaacggcaccgcgcagcccaacgacagttcgttcgtgcacctggtgacggcactgcgcgcgaacatgcccgacaagatcatcagcctctacaacatcggcccggccgcgtcccgcctgtcgtacggcggtgtcgacgtctccgacaagttcgactacgcctggaatccctactacggcacctggcaggtccccggcatcgcactgcccaaggcgcagctgtcgccggcggccgtcgagatcggccggacctcacggagcaccgtcgccgacctcgcccgtcgcaccgtcgacgaggggtacggcgtctatctgacgtacaacctcgacggcggcgatcgcaccgccgacgtctccgcgttcaccagggagctgtacggcagcgaggcggtccggacgccgtgataa

SEQ ID NO: 32 - DNA, 1248 bp, Artificial sequence
  synthetic DNA encoding His6-TnGalNAcT(33-421)
  sig_peptide (4)..(57)
atgaattttggactgaggctgattttcctggtgctgaccctgaaaggcgtccagtgtcatcaccatcaccatcactccccgcttcgcacatatctttacactccattatacaatgccacccagcccacactcagaaacgtcgagaggctggcagctaactggccaaagaagatccctagtaattatatagaagatagcgaagagtatagcatcaagaatatttctttgagcaaccacacaactagagcatctgtggtacatcctccttcctctatcaccgaaacggcaagcaaactggataagaatatgaccatccaagacggcgcctttgctatgattagcccgacgcccttgcttatcaccaaattgatggatagcatcaaatcttatgttactaccgaggatggggttaagaaagccgaagccgtcgtaactctccccctctgtgatagcatgcctcctgaccttggtcctattactcttaacaaaaccgagctcgagctcgaatgggttgagaaaaagttccctgaggtcgagtggggtggacgttatagtccccccaactgcacagctaggcatcgcgtagcaatcatagtcccgtaccgagacagacagcaacacctggcaatcttcttaaatcacatgcaccccttcctgatgaaacagcagatcgaatatggcatctttatcgtggagcaggaaggaaacaaggactttaaccgtgcgaaacttatgaacgtcggctttgttgaaagtcaaaaactcgttgccgagggatggcagtgtttcgtttttcatgacatagacctgctcccactggacactagaaacctctatagctgcccgagacagccacgccacatgagcgcttccattgacaaacttcactttaagctgccttacgaagacatcttcggtggcgtgtcagccatgactctggaacagttcacccgagtgaatggattttcaaataaatactggggatgggggggagaggacgacgatatgagttatcggcttaagaaaatcaactaccatattgcaagatataaaatgtccatcgcccgatacgccatgttggaccacaagaagtcaacacccaatcctaagcggtaccaattactctcacagacctcaaagacattccagaaagacgggctgagcaccctggaatatgagctggtgcaagtcgttcaatatcatctgtatactcacatcctggttaatattgacgagaggtcctgataa

SEQ ID NO: 33 - protein, 395 aa, Artificial sequence
  His6-TnGalNAcT(33-421)
HHHHHHSPLRTYLYTPLYNATQPTLRNVERLAANWPKKIPSNYIEDSEEYSIKNISLSNHTTRASVVHPPSSITETASKLDKNMTIQDGAFAMISPTPLLITKLMDSIKSYVTTEDGVKKAEAVVTLPLCDSMPPDLGPITLNKTELELEWVEKKFPEVEWGGRYSPPNCTARHRVAIIVPYRDRQQHLAIFLNHMHPFLMKQQIEYGIFIVEQEGNKDFNRAKLMNVGFVESQKLVAEGWQCFVFHDIDLLPLDTRNLYSCPRQPRHMSASIDKLHFKLPYEDIFGGVSAMTLEQFTRVNGFSNKYWGWGGEDDDMSYRLKKINYHIARYKMSIARYAMLDHKKSTPNPKRYQLLSQTSKTFQKDGLSTLEYELVQVVQYHLYTHILVNIDERS